European Patent Specification EP 3 824 907 B1, published September 17, 2025. Title: Therapeutic agent or prophylactic agent for HAM. Applicant: The University of Tokyo St. Marianna University School of Medicine. The sequence listing filed with the application follows.

SEQUENCE LISTING (109 sequences)

SEQ ID NO: 1 - DNA, 1299 bp, Homo sapiens
atggggagaggggcaggacgttcagccctgggattctggccgaccctcgccttccttctctgcagcttccccgcagccacctccccgtgcaagatcctcaagtgcaactctgagttctggagcgccacgtcgggcagccacgccccagcctcagacgacacccccgagttctgtgcagccttgcgcagctacgccctgtgcacgcggcggacggcccgcacctgccggggtgacctggcctaccactcggccgtccatggcatagaggacctcatgagccagcacaactgctccaaggatggccccacctcgcagccacgcctgcgcacgctcccaccggccggagacagccaggagcgctcggacagccccgagatctgccattacgagaagagctttcacaagcactcggccacccccaactacacgcactgtggcctcttcggggacccacacctcaggactttcaccgaccgcttccagacctgcaaggtgcagggcgcctggccgctcatcgacaataattacctgaacgtgcaggtcaccaacacgcctgtgctgcccggctcagcggccactgccaccagcaagctcaccatcatcttcaagaacttccaggagtgtgtggaccagaaggtgtaccaggctgagatggacgagctcccggccgccttcgtggatggctctaagaacggtggggacaagcacggggccaacagcctgaagatcactgagaaggtgtcaggccagcacgtggagatccaggccaagtacatcggcaccaccatcgtggtgcgccaggtgggccgctacctgacctttgccgtccgcatgccagaggaagtggtcaatgctgtggaggactgggacagccagggtctctacctctgcctgcggggctgccccctcaaccagcagatcgacttccaggccttccacaccaatgctgagggcaccggtgcccgcaggctggcagccgccagccctgcacccacagcccccgagaccttcccatacgagacagccgtggccaagtgcaaggagaagctgccggtggaggacctgtactaccaggcctgcgtcttcgacctcctcaccacgggcgacgtgaacttcacactggccgcctactacgcgttggaggatgtcaagatgctccactccaacaaagacaaactgcacctgtatgagaggactcgggacctgccaggcagggcggctgcggggctgcccctggccccccggcccctcctgggcgccctcgtcccgctcctggccctgctccctgtgttctgctag

SEQ ID NO: 2 - DNA, 1296 bp, Rattus norvegicus
atggggagaggggcaggacgttcagccctgggattgtggccgaccctcgccttccttctctgcagctttcccgcagctatctctccctgcaagatcctcaagtgcaactctgagttctggagcgccacgtcgtcaggcagccacgcccctgcctctgacgacgtgcccgagttctgtgctgccctgcgcacctacgccctgtgcacgcgacggacagcccgcacctgccggggcgacctggcttaccactcggctgtccatggcatagaggacctcatgagccagcacaactgctccaaggatggccccacctcacagcctcgagtgcgcacgctcccgccagctggggacagccaggagcgctcagatagccccgagatctgccactatgagaagagtttccacaagcactcagctgcccccaactacactcactgcggcctctttggggacccacacctcaggactttcacagaccacttccagacatgtaaggtgcaaggcgcttggcctctcatcgacaataattacctgaacgtgcaggtcaccaatacacctgtgctgcccggctctgccgccactgccaccagcaagctcaccatcatcttcaagaacttccaagagtgtgtggaccagaaagtataccaagccgagatggacgagcttccgtccgcctttgccgatggctccaaaaacggtggagataaacacggagccaacagcctgaagatcacagagaaggtgtcaggccagcacgtggagatccaggccaagtacatcggcaccaccatcgtggtgagacaggtgggccgctacctgaccttcgccgtccggatgcccgaggaggtagtcaacgccgtggaggaccgtgacagccaaggcctctacctctgcctgcggggctgcccgctcaaccagcagatcgacttccaggctttccgtgccaacgccgagagccctcgcaggccagcagctgccagcccctctcctgtggtccccgagacatttccgtacgagacagctgtggccaagtgcaaagagaagctgcctgtagaagacttgtactaccaggcctgtgtcttcgacctcctcacgactggcgacgtgaacttcacgctggccgcctactatgctttggaggatggcaagatgctccactccaacaaggacaagctacacctgtttgaaaggactcgggagctgcctggcgctgtggccgctgcagcatttcccttggcccccgagatgctcccgggcaccgtcacacttctggtcctgctgcctctgttctggtag

SEQ ID NO: 3 - protein, 432 aa, Homo sapiens
MGRGAGRSALGFWPTLAFLLCSFPAATSPCKILKCNSEFWSATSGSHAPASDDTPEFCAALRSYALCTRRTARTCRGDLAYHSAVHGIEDLMSQHNCSKDGPTSQPRLRTLPPAGDSQERSDSPEICHYEKSFHKHSATPNYTHCGLFGDPHLRTFTDRFQTCKVQGAWPLIDNNYLNVQVTNTPVLPGSAATATSKLTIIFKNFQECVDQKVYQAEMDELPAAFVDGSKNGGDKHGANSLKITEKVSGQHVEIQAKYIGTTIVVRQVGRYLTFAVRMPEEVVNAVEDWDSQGLYLCLRGCPLNQQIDFQAFHTNAEGTGARRLAAASPAPTAPETFPYETAVAKCKEKLPVEDLYYQACVFDLLTTGDVNFTLAAYYALEDVKMLHSNKDKLHLYERTRDLPGRAAAGLPLAPRPLLGALVPLLALLPVFC

SEQ ID NO: 4 - protein, 431 aa, Rattus norvegicus
MGRGAGRSALGLWPTLAFLLCSFPAAISPCKILKCNSEFWSATSSGSHAPASDDVPEFCAALRTYALCTRRTARTCRGDLAYHSAVHGIEDLMSQHNCSKDGPTSQPRVRTLPPAGDSQERSDSPEICHYEKSFHKHSAAPNYTHCGLFGDPHLRTFTDHFQTCKVQGAWPLIDNNYLNVQVTNTPVLPGSAATATSKLTIIFKNFQECVDQKVYQAEMDELPSAFADGSKNGGDKHGANSLKITEKVSGQHVEIQAKYIGTTIVVRQVGRYLTFAVRMPEEVVNAVEDRDSQGLYLCLRGCPLNQQIDFQAFRANAESPRRPAAASPSPVVPETFPYETAVAKCKEKLPVEDLYYQACVFDLLTTGDVNFTLAAYYALEDGKMLHSNKDKLHLFERTRELPGAVAAAAFPLAPEMLPGTVTLLVLLPLFW

SEQ ID NO: 5 - protein, 5 aa, Artificial
  VH 5F9 CDR H1
NYGMN

SEQ ID NO: 6 - protein, 17 aa, Artificial
  VH 5F9 CDR-H2
MIYYDSSEKHYADSVKG

SEQ ID NO: 7 - protein, 6 aa, Artificial
  VH 5F9 CDR-H3
GTTPDY

SEQ ID NO: 8 - protein, 16 aa, Artificial
  VL 5F9 CDR-L1
RSSQSLEYSDGYTFLE

SEQ ID NO: 9 - protein, 7 aa, Artificial
  VL 5F9 CDR-L2
EVSNRFS

SEQ ID NO: 10 - protein, 9 aa, Artificial
  VL 5F9 CDR-L3
FQATHDPLT

SEQ ID NO: 11 - protein, 5 aa, Artificial
  VH 8D1 CDR-H1
SYVMH

SEQ ID NO: 12 - protein, 17 aa, Artificial
  VH 8D1 CDR-H2
YIIPYNDNTKYNEKFKG

SEQ ID NO: 13 - protein, 14 aa, Artificial
  VH 8D1 CDR-H3
ARRNEYYGSSFFDY

SEQ ID NO: 14 - protein, 11 aa, Artificial
  VL 8D1 CDR-L1
QASQDIDNYLA

SEQ ID NO: 15 - protein, 7 aa, Artificial
  VL 8D1 CDR-L2
GATNLAD

SEQ ID NO: 16 - protein, 9 aa, Artificial
  VL 8D1 CDR-L3
LQGYIPPRT

SEQ ID NO: 17 - protein, 115 aa, Artificial
  VH 5F9
EVQLVESGGGLVQPGSSLKLSCVASGFTFSNYGMNWIRQAPKKGLEWIGMIYYDSSEKHYADSVKGRFTISRDNSKNTLYLEMNSLRSEDTAIYYCAKGTTPDYWGQGVMVTVSS

SEQ ID NO: 18 - protein, 113 aa, Artificial
  VL 5F9
DVVLTQTPVSLSVTLGDQASMSCRSSQSLEYSDGYTFLEWFLQKPGQSPQLLIYEVSNRFSGVPDRFIGSGSGTDFTLKISRVEPEDLGVYYCFQATHDPLTFGSGTKLEIKR

SEQ ID NO: 19 - protein, 121 aa, Artificial
  VH 8D1
EVQLQQSGPELVKPGTSVKMSCKTSGYTFTSYVMHWVKQKPGQGLEWIGYIIPYNDNTKYNEKFKGKATLTSDKSSSTAYMELSSLTSEDSAVYYCARRNEYYGSSFFDYWGQGTTLTVSS

SEQ ID NO: 20 - protein, 108 aa, Artificial
  VL 8D1
DIQMTQSPASLSASLEEIVTITCQASQDIDNYLAWYHQKPGKSPRLLIYGATNLADGVPSRFSGSRSGTQFSLKINRLQIEDLGIYYCLQGYIPPRTFGGGTKLELKR

SEQ ID NO: 21 - protein, 5 aa, Artificial
  VH 5F9 CDR H1
NYGMN

SEQ ID NO: 22 - protein, 30 aa, Artificial
  VH3-48/JH3 FR1
EVQLVESGGGLVQPGGSLRLSCAASGFTFS

SEQ ID NO: 23 - protein, 14 aa, Artificial
  VH3-48/JH3 FR2
WVRQAPGKGLEWVS

SEQ ID NO: 24 - protein, 32 aa, Artificial
  VH3-48/JH3 FR3
RFTISRDNAKNSLYLQMNSLRDEDTAVYYCAR

SEQ ID NO: 25 - protein, 11 aa, Artificial
  VH3-49/JH3 FR4
WGQGTMVTVSS

SEQ ID NO: 26 - protein, 11 aa, Artificial
  VH3-48/JH4 FR4
WGQGTLVTVSS

SEQ ID NO: 27 - protein, 11 aa, Artificial
  VH3-48/JH6 FR4
WGQGTTVTVSS

SEQ ID NO: 28 - protein, 30 aa, Artificial
  VH3-33/JH6 FR!
QVQLVESGGGVVQPGRSLRLSCAASGFTFS

SEQ ID NO: 29 - protein, 14 aa, Artificial
  VH3-33/JH6 FR2
WVRQAPGKGLEWVA

SEQ ID NO: 30 - protein, 32 aa, Artificial
  VH3-33/JH6 FR3
RFTISRDNSKNTLYLQMNSLRAEDTAVYYCAR

SEQ ID NO: 31 - protein, 30 aa, Artificial
  VH3-23/JH3 FR1
EVQLLESGGGLVQPGGSLRLSCAASGFTFS

SEQ ID NO: 32 - protein, 14 aa, Artificial
  VH3-23/JH3 FR2
WVRQAPGKGLEWVS

SEQ ID NO: 33 - protein, 32 aa, Artificial
  VH3-23/JH3 FR3
RFTISRDNSKNTLYLQMNSLRAEDTAVYYCAK

SEQ ID NO: 34 - protein, 23 aa, Artificial
  A18/JK2 FR1
DIVMTQTPLSLSVTPGQPASISC

SEQ ID NO: 35 - protein, 15 aa, Artificial
  A18/JK2 FR2
WYLQKPGQSPQLLIY

SEQ ID NO: 36 - protein, 32 aa, Artificial
  A18/JK2 FR3
GVPDRFSGSGSGTDFTLKISRVEAEDVGVYYC

SEQ ID NO: 37 - protein, 11 aa, Artificial
  A18/JK2 FR4
FGQGTKLEIKR

SEQ ID NO: 38 - protein, 23 aa, Artificial
  A17/JK2 FR1
DVVMTQSPLSLPVTLGQPASISC

SEQ ID NO: 39 - protein, 15 aa, Artificial
  A17/JK2 FR2
WFQQRPGQSPRRLIY

SEQ ID NO: 40 - protein, 32 aa, Artificial; identical to SEQ ID NO: 36
  A17/JK2 FR3

SEQ ID NO: 41 - protein, 115 aa, Artificial
  VH 5F9.1-GL
EVQLVESGGGLVQPGGSLRLSCAASGFTFSNYGMNWVRQAPGKGLEWVSMIYYDSSEKHYADSVKGRFTISRDNAKNSLYLQMNSLRDEDTAVYYCARGTTPDYWGQGTMVTVSS

SEQ ID NO: 42 - protein, 115 aa, Artificial
  VH 5F9.2-GL
EVQLVESGGGLVQPGGSLRLSCAASGFTFSNYGMNWVRQAPGKGLEWVSMIYYDSSEKHYADSVKGRFTISRDNAKNSLYLQMNSLRDEDTAVYYCARGTTPDYWGQGTLVTVSS

SEQ ID NO: 43 - protein, 115 aa, Artificial
  VH 5F9.3-GL
EVQLVESGGGLVQPGGSLRLSCAASGFTFSNYGMNWVRQAPGKGLEWVSMIYYDSSEKHYADSVKGRFTISRDNAKNSLYLQMNSLRDEDTAVYYCARGTTPDYWGQGTTVTVSS

SEQ ID NO: 44 - protein, 115 aa, Artificial
  VH 5F9.4-GL
QVQLVESGGGVVQPGRSLRLSCAASGFTFSNYGMNWVRQAPGKGLEWVAMIYYDSSEKHYADSVKGRFTISRDNSKNTLYLQMNSLRAEDTAVYYCARGTTPDYWGQGTMVTVSS

SEQ ID NO: 45 - protein, 115 aa, Artificial
  VH 5F9.5-GL
QVQLVESGGGVVQPGRSLRLSCAASGFTFSNYGMNWVRQAPGKGLEWVAMIYYDSSEKHYADSVKGRFTISRDNSKNTLYLQMNSLRAEDTAVYYCARGTTPDYWGQGTLVTVSS

SEQ ID NO: 46 - protein, 115 aa, Artificial
  VH 5F9.6-GL
QVQLVESGGGVVQPGRSLRLSCAASGFTFSNYGMNWVRQAPGKGLEWVAMIYYDSSEKHYADSVKGRFTISRDNSKNTLYLQMNSLRAEDTAVYYCARGTTPDYWGQGTTVTVSS

SEQ ID NO: 47 - protein, 115 aa, Artificial
  VH 5F9.7-GL
EVQLLESGGGLVQPGGSLRLSCAASGFTFSNYGMNWVRQAPGKGLEWVSMIYYDSSEKHYADSVKGRFTISRDNSKNTLYLQMNSLRAEDTAVYYCAKGTTPDYWGQGTMVTVSS

SEQ ID NO: 48 - protein, 115 aa, Artificial
  VH 5F9.8-GL
EVQLLESGGGLVQPGGSLRLSCAASGFTFSNYGMNWVRQAPGKGLEWVSMIYYDSSEKHYADSVKGRFTISRDNSKNTLYLQMNSLRAEDTAVYYCAKGTTPDYWGQGTLVTVSS

SEQ ID NO: 49 - protein, 115 aa, Artificial
  VH 5F9.9-GL
EVQLLESGGGLVQPGGSLRLSCAASGFTFSNYGMNWVRQAPGKGLEWVSMIYYDSSEKHYADSVKGRFTISRDNSKNTLYLQMNSLRAEDTAVYYCAKGTTPDYWGQGTTVTVSS

SEQ ID NO: 50 - protein, 113 aa, Artificial
  VL 5F9.1-GL
DIVMTQTPLSLSVTPGQPASISCRSSQSLEYSDGYTFLEWYLQKPGQSPQLLIYEVSNRFSGVPDRFSGSGSGTDFTLKISRVEAEDVGVYYCFQATHDPLTFGQGTKLEIKR

SEQ ID NO: 51 - protein, 113 aa, Artificial
  VL 5F9.2-GL
DVVMTQSPLSLPVTLGQPASISCRSSQSLEYSDGYTFLEWFQQRPGQSPRRLIYEVSNRFSGVPDRFSGSGSGTDFTLKISRVEAEDVGVYYCFQATHDPLTFGQGTKLEIKR

SEQ ID NO: 52 - protein, 113 aa, Artificial
  VL 5F9.3-GL
DVVMTQSPLSLPVTLGQPASISCRSSQSLEYSDGYTFLEWYLQKPGQSPQLLIYEVSNRFSGVPDRFSGSGSGTDFTLKISRVEAEDVGVYYCFQATHDPLTFGQGTKLEIKR

SEQ ID NO: 53 - protein, 14 aa, Mus musculus
EEVVNAVEDWDSQG

SEQ ID NO: 54 - protein, 14 aa, Mus musculus
NQQIDFQAFHTNAE

SEQ ID NO: 55 - protein, 11 aa, Mus musculus
PTAPETFPYET

SEQ ID NO: 56 - protein, 11 aa, Mus musculus
KLPVEDLYYQA

SEQ ID NO: 57 - protein, 16 aa, Homo sapiens
LYERTRDLPGRAAAGL

SEQ ID NO: 58 - protein, 11 aa, Mus musculus
RASQDISSYLN

SEQ ID NO: 59 - protein, 7 aa, Mus musculus
YTSRLHS

SEQ ID NO: 60 - protein, 7 aa, Mus musculus
QQLNTLP

SEQ ID NO: 61 - protein, 5 aa, Mus musculus
DAWMD

SEQ ID NO: 62 - protein, 19 aa, Mus musculus
EIRSKANNHATYYAESVKG

SEQ ID NO: 63 - protein, 5 aa, Mus musculus
RDGAY

SEQ ID NO: 64 - protein, 16 aa, Mus musculus
RSSQSLVHSNGNTYLH

SEQ ID NO: 65 - protein, 7 aa, Mus musculus
KVSNRFS

SEQ ID NO: 66 - protein, 7 aa, Mus musculus
SQSTHVP

SEQ ID NO: 67 - protein, 6 aa, Mus musculus
TSYYWN

SEQ ID NO: 68 - protein, 16 aa, Mus musculus
YISYDGTNNYNPSLKN

SEQ ID NO: 69 - skipped

SEQ ID NO: 70 - protein, 450 aa, Homo sapiens
MQPPRERLVVTGRAGWMGMGRGAGRSALGFWPTLAFLLCSFPAATSPCKILKCNSEFWSATSGSHAPASDDTPEFCAALRSYALCTRRTARTCRGDLAYHSAVHGIEDLMSQHNCSKDGPTSQPRLRTLPPAGDSQERSDSPEICHYEKSFHKHSATPNYTHCGLFGDPHLRTFTDRFQTCKVQGAWPLIDNNYLNVQVTNTPVLPGSAATATSKLTIIFKNFQECVDQKVYQAEMDELPAAFVDGSKNGGDKHGANSLKITEKVSGQHVEIQAKYIGTTIVVRQVGRYLTFAVRMPEEVVNAVEDWDSQGLYLCLRGCPLNQQIDFQAFHTNAEGTGARRLAAASPAPTAPETFPYETAVAKCKEKLPVEDLYYQACVFDLLTTGDVNFTLAAYYALEDVKMLHSNKDKLHLYDRTRDLPGRAAAGLPLAPRPLLGALVPLLALLPVFC

SEQ ID NO: 71 - protein, 454 aa, Mus musculus
MQPPRERLVVTGRAGWMGMGRGAGRSALGLWPTLAFLLCSFPAAISPCKILKCNSEFWSATSSGSHAPASDDVPEFCAALRTYALCTRRTARTCRGDLAYHSAVHGIEDLMSQHNCSKDGPTSQPRVRTLPPAGDSQERSDSPEICHYEKSFHKHSAAPNYTHCGLFGDPHLRTFTDHFQTCKVQGAWPLIDNNYLNVQVTNTPVLPGSAATATSKLTIIFKNFQECVDQKVYQAEMDELPSAFADGSKNGGDKHGANSLKITEKVSGQHVEIQAKYIGTTIVVRQVGRYLTFAVRMPEEVVNAVEDRDSQGLYLCLRGCPLNQQIDFQAFRANAESPRRPAAASPSPVVPETFPYETAVAKCKEKLPVEDLYYQACVFDLLTTGDVNFTLAAYYALEDGKMLHSNKDKLHLFERTRELPGAVAAAAAAATTFPLAPQILLGTIPLLVLLPVLW

SEQ ID NO: 72 - protein, 449 aa, Rattus norvegicus
MQPPRERLVVTGRAGWMGMGRGAGRSALGLWPTLAFLLCSFPAAISPCKILKCNSEFWSATSSGSHAPASDDVPEFCAALRTYALCTRRTARTCRGDLAYHSAVHGIEDLMSQHNCSKDGPTSQPRVRTLPPAGDSQERSDSPEICHYEKSFHKHSAAPNYTHCGLFGDPHLRTFTDHFQTCKVQGAWPLIDNNYLNVQVTNTPVLPGSAATATSKLTIIFKNFQECVDQKVYQAEMDELPSAFADGSKNGGDKHGANSLKITEKVSGQHVEIQAKYIGTTIVVRQVGRYLTFAVRMPEEVVNAVEDRDSQGLYLCLRGCPLNQQIDFQAFRANAESPRRPAAASPSPVVPETFPYETAVAKCKEKLPVEDLYYQACVFDLLTTGDVNFTLAAYYALEDGKMLHSNKDKLHLFERTRELPGAVAAAAFPLAPEMLPGTVTLLVLLPLFW

SEQ ID NO: 73 - protein, 234 aa, Mus musculus
MMSSAQFLGLLLLCFQGTRCDIQMTQTTSSLSASLGDRVTISCRASQDISSYLNWYQQKPDGTVKLLIYYTSRLHSGVPSRFSGSGSGTDYSLTISNLEQEDIATYFCQQLNTLPWTFGGGTKLEIKRADAAPTVSIFPPSSEQLTSGGASVVCFLNNFYPKDINVKWKIDGSERQNGVLNSWTDQDSKDSTYSMSSTLTLTKDEYERHNSYTCEATHKTSTSPIVKSFNRNEC

SEQ ID NO: 74 - protein, 471 aa, Mus musculus
MYLGLNYVFIVFLLNGVQSEVKLEESGGGLVQPGGSMKLSCAASGFTFSDAWMDWVRQSPEKGLEWVAEIRSKANNHATYYAESVKGRFTISRDDSKRSVYLQMNNLRAEDTGIYYCTRRDGAYWGQGTLVTVSAAKTTPPSVYPLAPGCGDTTGSSVTLGCLVKGYFPESVTVTWNSGSLSSSVHTFPALLQSGLYTMSSSVTVPSSTWPSQTVTCSVAHPASSTTVDKKLEPSGPISTINPCPPCKECHKCPAPNLEGGPSVFIFPPNIKDVLMISLTPKVTCVVVDVSEDDPDVQISWFVNNVEVHTAQTQTHREDYNSTIRVVSTLPIQHQDWMSGKEFKCKVNNKDLPSPIERTISKIKGLVRAPQVYILPPPAEQLSRKDVSLTCLVVGFNPGDISVEWTSNGHTEENYKDTAPVLDSDGSYFIYSKLNMKTSKWEKTDSFSCNVRHEGLKNYYLKKTISRSPGK

SEQ ID NO: 75 - protein, 238 aa, Mus musculus
MKLPVRLLVLMFWIPASSSDVVMTQTPLSLPVSLGDQASISCRSSQSLVHSNGNTYLHWYLQRPGQSPKLLIYKVSNRFSGVPDRFSGSGSGTDFTLKISRVEAEDLGLYFCSQSTHVPYTFGGGTKLEIKRADAAPTVSIFPPSSEQLTSGGASVVCFLNNFYPKDINVKWKIDGSERQNGVLNSWTDQDSKDSTYSMSSTLTLTKDEYERHNSYTCEATHKTSTSPIVKSFNRNEC

SEQ ID NO: 76 - protein, 466 aa, Mus musculus
MKVLSLLYLLTAIPGIMSDVKLQESGPGLVKPSQSLSLTCSVTGYSITTSYYWNWIRQFPGNKLEWMGYISYDGTNNYNPSLKNRISITRDTSKNQFFLRLNSVTTEDTATYYCAGSFGYSQGTLVTVSAAKTTPPSVYPLAPGCGDTTGSSVTLGCLVKGYFPESVTVTWNSGSLSSSVHTFPALLQSGLYTMSSSVTVPSSTWPSQTVTCSVAHPASSTTVDKKLEPSGPISTINPCPPCKECHKCPAPNLEGGPSVFIFPPNIKDVLMISLTPKVTCVVVDVSEDDPDVQISWFVNNVEVHTAQTQTHREDYNSTIRVVSTLPIQHQDWMSGKEFKCKVNNKDLPSPIERTISKIKGLVRAPQVYILPPPAEQLSRKDVSLTCLVVGFNPGDISVEWTSNGHTEENYKDTAPVLDSDGSYFIYSKLNMKTSKWEKTDSFSCNVRHEGLKNYYLKKTISRSPGK

SEQ ID NO: 77 - protein, 214 aa, Artificial Sequence
  chimeric antibody light chain
DIQMTQTTSSLSASLGDRVTISCRASQDISSYLNWYQQKPDGTVKLLIYYTSRLHSGVPSRFSGSGSGTDYSLTISNLEQEDIATYFCQQLNTLPWTFGGGTKLEIKRTVAAPSVFIFPPSDEQLKSGTASVVCLLNNFYPREAKVQWKVDNALQSGNSQESVTEQDSKDSTYSLSSTLTLSKADYEKHKVYACEVTHQGLSSPVTKSFNRGEC

SEQ ID NO: 78 - protein, 446 aa, Artificial Sequence
  chimeric antibody heavy chain
EVKLEESGGGLVQPGGSMKLSCAASGFTFSDAWMDWVRQSPEKGLEWVAEIRSKANNHATYYAESVKGRFTISRDDSKRSVYLQMNNLRAEDTGIYYCTRRDGAYWGQGTLVTVSAASTKGPSVFPLAPSSKSTSGGTAALGCLVKDYFPEPVTVSWNSGALTSGVHTFPAVLQSSGLYSLSSVVTVPSSSLGTQTYICNVNHKPSNTKVDKKVEPKSCDKTHTCPPCPAPELLGGPSVFLFPPKPKDTLMISRTPEVTCVVVDVSHEDPEVKFNWYVDGVEVHNAKTKPREEQYNSTYRVVSVLTVLHQDWLNGKEYKCKVSNKALPAPIEKTISKAKGQPREPQVYTLPPSRDELTKNQVSLTCLVKGFYPSDIAVEWESNGQPENNYKTTPPVLDSDGSFFLYSKLTVDKSRWQQGNVFSCSVMHEALHNHYTQKSLSLSPGK

SEQ ID NO: 79 - protein, 1461 aa, Homo sapiens
MAAERGARRLLSTPSFWLYCLLLLGRRAPGAAAARSGSAPQSPGASIRTFTPFYFLVEPVDTLSVRGSSVILNCSAYSEPSPKIEWKKDGTFLNLVSDDRRQLLPDGSLFISNVVHSKHNKPDEGYYQCVATVESLGTIISRTAKLIVAGLPRFTSQPEPSSVYAGNNAILNCEVNADLVPFVRWEQNRQPLLLDDRVIKLPSGMLVISNATEGDGGLYRCVVESGGPPKYSDEVELKVLPDPEVISDLVFLKQPSPLVRVIGQDVVLPCVASGLPTPTIKWMKNEEALDTESSERLVLLAGGSLEISDVTEDDAGTYFCIADNGNETIEAQAELTVQAQPEFLKQPTNIYAHESMDIVFECEVTGKPTPTVKWVKNGDMVIPSDYFKIVKEHNLQVLGLVKSDEGFYQCIAENDVGNAQAGAQLIILEHAPATTGPLPSAPRDVVASLVSTRFIKLTWRTPASDPHGDNLTYSVFYTKEGIARERVENTSHPGEMQVTIQNLMPATVYIFRVMAQNKHGSGESSAPLRVETQPEVQLPGPAPNLRAYAASPTSITVTWETPVSGNGEIQNYKLYYMEKGTDKEQDVDVSSHSYTINGLKKYTEYSFRVVAYNKHGPGVSTPDVAVRTLSDVPSAAPQNLSLEVRNSKSIMIHWQPPAPATQNGQITGYKIRYRKASRKSDVTETLVSGTQLSQLIEGLDRGTEYNFRVAALTINGTGPATDWLSAETFESDLDETRVPEVPSSLHVRPLVTSIVVSWTPPENQNIVVRGYAIGYGIGSPHAQTIKVDYKQRYYTIENLDPSSHYVITLKAFNNVGEGIPLYESAVTRPHTDTSEVDLFVINAPYTPVPDPTPMMPPVGVQASILSHDTIRITWADNSLPKHQKITDSRYYTVRWKTNIPANTKYKNANATTLSYLVTGLKPNTLYEFSVMVTKGRRSSTWSMTAHGTTFELVPTSPPKDVTVVSKEGKPKTIIVNWQPPSEANGKITGYIIYYSTDVNAEIHDWVIEPVVGNRLTHQIQELTLDTPYYFKIQARNSKGMGPMSEAVQFRTPKADSSDKMPNDQASGSGGKGSRLPDLGSDYKPPMSGSNSPHGSPTSPLDSNMLLVIIVSVGVITIVVVVIIAVFCTRRTTSHQKKKRAACKSVNGSHKYKGNSKDVKPPDLWIHHERLELKPIDKSPDPNPIMTDTPIPRNSQDITPVDNSMDSNIHQRRNSYRGHESEDSMSTLAGRRGMRPKMMMPFDSQPPQPVISAHPIHSLDNPHHHFHSSSLASPARSHLYHPGSPWPIGTSMSLSDRANSTESVRNTPSTDTMPASSSQTCCTDHQDPEGATSSSYLASSQEEDSGQSLPTAHVRPSHPLKSFAVPAIPPPGPPTYDPALPSTPLLSQQALNHHIHSVKTASIGTLGRSRPPMPVVVPSAPEVQETTRMLEDSESSYEPDELTKEMAHLEGLMKDLNAITTA

SEQ ID NO: 80 - protein, 446 aa, Artificial Sequence
  humanized antibody heavy chain HA
EVQLVESGGGLVQPGRSLRLSCTASGFTFSDAWMDWFRQAPGKGLEWVAEIRSKANNHATYYAESVKGRFTISRDDSKSIAYLQMNSLKTEDTALYYCTRRDGAYWGKGTTVTVSSASTKGPSVFPLAPSSKSTSGGTAALGCLVKDYFPEPVTVSWNSGALTSGVHTFPAVLQSSGLYSLSSVVTVPSSSLGTQTYICNVNHKPSNTKVDKKVEPKSCDKTHTCPPCPAPELLGGPSVFLFPPKPKDTLMISRTPEVTCVVVDVSHEDPEVKFNWYVDGVEVHNAKTKPREEQYNSTYRVVSVLTVLHQDWLNGKEYKCKVSNKALPAPIEKTISKAKGQPREPQVYTLPPSRDELTKNQVSLTCLVKGFYPSDIAVEWESNGQPENNYKTTPPVLDSDGSFFLYSKLTVDKSRWQQGNVFSCSVMHEALHNHYTQKSLSLSPGK

SEQ ID NO: 81 - protein, 446 aa, Artificial Sequence
  humanized antibody heavy chain HB
EVQLVESGGGLVQPGRSLRLSCTASGFTFSDAWMDWFRQAPGKGLEWVAEIRSKANNHATYYAESVKGRFTISRDDSKSIVYLQMNSLRTEDTALYYCTRRDGAYWGKGTTVTVSSASTKGPSVFPLAPSSKSTSGGTAALGCLVKDYFPEPVTVSWNSGALTSGVHTFPAVLQSSGLYSLSSVVTVPSSSLGTQTYICNVNHKPSNTKVDKKVEPKSCDKTHTCPPCPAPELLGGPSVFLFPPKPKDTLMISRTPEVTCVVVDVSHEDPEVKFNWYVDGVEVHNAKTKPREEQYNSTYRVVSVLTVLHQDWLNGKEYKCKVSNKALPAPIEKTISKAKGQPREPQVYTLPPSRDELTKNQVSLTCLVKGFYPSDIAVEWESNGQPENNYKTTPPVLDSDGSFFLYSKLTVDKSRWQQGNVFSCSVMHEALHNHYTQKSLSLSPGK

SEQ ID NO: 82 - protein, 446 aa, Artificial Sequence
  humanized antibody heavy chain HC
EVQLVESGGGLVQPGRSLRLSCTASGFTFSDAWMDWFRQAPGKGLEWVAEIRSKANNHATYYAESVKGRFTISRDDSKSIVYLQMNSLKTEDTALYYCTRRDGAYWGKGTTVTVSSASTKGPSVFPLAPSSKSTSGGTAALGCLVKDYFPEPVTVSWNSGALTSGVHTFPAVLQSSGLYSLSSVVTVPSSSLGTQTYICNVNHKPSNTKVDKKVEPKSCDKTHTCPPCPAPELLGGPSVFLFPPKPKDTLMISRTPEVTCVVVDVSHEDPEVKFNWYVDGVEVHNAKTKPREEQYNSTYRVVSVLTVLHQDWLNGKEYKCKVSNKALPAPIEKTISKAKGQPREPQVYTLPPSRDELTKNQVSLTCLVKGFYPSDIAVEWESNGQPENNYKTTPPVLDSDGSFFLYSKLTVDKSRWQQGNVFSCSVMHEALHNHYTQKSLSLSPGK

SEQ ID NO: 83 - protein, 446 aa, Artificial Sequence
  humanized antibody heavy chain HD
EVQLVESGGGLVQPGRSLRLSCTASGFTFSDAWMDWFRQAPGKGLEWVAEIRSKANNHATYYAESVKGRFTISRDDSKSIAYLQMNSLRTEDTALYYCTRRDGAYWGKGTTVTVSSASTKGPSVFPLAPSSKSTSGGTAALGCLVKDYFPEPVTVSWNSGALTSGVHTFPAVLQSSGLYSLSSVVTVPSSSLGTQTYICNVNHKPSNTKVDKKVEPKSCDKTHTCPPCPAPELLGGPSVFLFPPKPKDTLMISRTPEVTCVVVDVSHEDPEVKFNWYVDGVEVHNAKTKPREEQYNSTYRVVSVLTVLHQDWLNGKEYKCKVSNKALPAPIEKTISKAKGQPREPQVYTLPPSRDELTKNQVSLTCLVKGFYPSDIAVEWESNGQPENNYKTTPPVLDSDGSFFLYSKLTVDKSRWQQGNVFSCSVMHEALHNHYTQKSLSLSPGK

SEQ ID NO: 84 - protein, 446 aa, Artificial Sequence
  humanized antibody heavy chain HE
EVQLVESGGGLVQPGRSLRLSCTASGFTFSDAWMDWVRQAPGKGLEWVAEIRSKANNHATYYAESVKGRFTISRDDSKSIVYLQMNSLRTEDTALYYCTRRDGAYWGKGTTVTVSSASTKGPSVFPLAPSSKSTSGGTAALGCLVKDYFPEPVTVSWNSGALTSGVHTFPAVLQSSGLYSLSSVVTVPSSSLGTQTYICNVNHKPSNTKVDKKVEPKSCDKTHTCPPCPAPELLGGPSVFLFPPKPKDTLMISRTPEVTCVVVDVSHEDPEVKFNWYVDGVEVHNAKTKPREEQYNSTYRVVSVLTVLHQDWLNGKEYKCKVSNKALPAPIEKTISKAKGQPREPQVYTLPPSRDELTKNQVSLTCLVKGFYPSDIAVEWESNGQPENNYKTTPPVLDSDGSFFLYSKLTVDKSRWQQGNVFSCSVMHEALHNHYTQKSLSLSPGK

SEQ ID NO: 85 - protein, 446 aa, Artificial Sequence
  humanized antibody heavy chain HF
EVQLVESGGGLVQPGRSLRLSCTASGFTFSDAWMDWFRQAPGKGLEWVAEIRSKANNHATYYAESVKGRFTISRDDSKSIAYLQMNSLKTEDTAVYYCTRRDGAYWGKGTTVTVSSASTKGPSVFPLAPSSKSTSGGTAALGCLVKDYFPEPVTVSWNSGALTSGVHTFPAVLQSSGLYSLSSVVTVPSSSLGTQTYICNVNHKPSNTKVDKKVEPKSCDKTHTCPPCPAPELLGGPSVFLFPPKPKDTLMISRTPEVTCVVVDVSHEDPEVKFNWYVDGVEVHNAKTKPREEQYNSTYRVVSVLTVLHQDWLNGKEYKCKVSNKALPAPIEKTISKAKGQPREPQVYTLPPSRDELTKNQVSLTCLVKGFYPSDIAVEWESNGQPENNYKTTPPVLDSDGSFFLYSKLTVDKSRWQQGNVFSCSVMHEALHNHYTQKSLSLSPGK

SEQ ID NO: 86 - protein, 446 aa, Artificial Sequence
  humanized antibody heavy chain HG
EVQLVESGGGLVQPGRSLRLSCTASGFTFSDAWMDWVRQAPGKGLEWVAEIRSKANNHATYYAESVKGRFTISRDDSKSIAYLQMNSLKTEDTALYYCTRRDGAYWGKGTTVTVSSASTKGPSVFPLAPSSKSTSGGTAALGCLVKDYFPEPVTVSWNSGALTSGVHTFPAVLQSSGLYSLSSVVTVPSSSLGTQTYICNVNHKPSNTKVDKKVEPKSCDKTHTCPPCPAPELLGGPSVFLFPPKPKDTLMISRTPEVTCVVVDVSHEDPEVKFNWYVDGVEVHNAKTKPREEQYNSTYRVVSVLTVLHQDWLNGKEYKCKVSNKALPAPIEKTISKAKGQPREPQVYTLPPSRDELTKNQVSLTCLVKGFYPSDIAVEWESNGQPENNYKTTPPVLDSDGSFFLYSKLTVDKSRWQQGNVFSCSVMHEALHNHYTQKSLSLSPGK

SEQ ID NO: 87 - protein, 446 aa, Artificial Sequence
  humanized antibody heavy chain HH
EVQLVESGGGLVQPGRSLRLSCTASGFTFSDAWMDWVRQAPGKGLEWVAEIRSKANNHATYYAESVKGRFTISRDDSKSIAYLQMNSLKTEDTAVYYCTRRDGAYWGKGTTVTVSSASTKGPSVFPLAPSSKSTSGGTAALGCLVKDYFPEPVTVSWNSGALTSGVHTFPAVLQSSGLYSLSSVVTVPSSSLGTQTYICNVNHKPSNTKVDKKVEPKSCDKTHTCPPCPAPELLGGPSVFLFPPKPKDTLMISRTPEVTCVVVDVSHEDPEVKFNWYVDGVEVHNAKTKPREEQYNSTYRVVSVLTVLHQDWLNGKEYKCKVSNKALPAPIEKTISKAKGQPREPQVYTLPPSRDELTKNQVSLTCLVKGFYPSDIAVEWESNGQPENNYKTTPPVLDSDGSFFLYSKLTVDKSRWQQGNVFSCSVMHEALHNHYTQKSLSLSPGK

SEQ ID NO: 88 - protein, 214 aa, Artificial Sequence
  humanized antibody light chain KA
DIQMTQSPSSVSASVGDRVTITCRASQDISSYLNWYQQKPGKAPKLLIYYTSRLHSGVPSRFSGSGSGTDFTLTISSLQPEDFASYFCQQLNTLPWTFGGGTKVEMERTVAAPSVFIFPPSDEQLKSGTASVVCLLNNFYPREAKVQWKVDNALQSGNSQESVTEQDSKDSTYSLSSTLTLSKADYEKHKVYACEVTHQGLSSPVTKSFNRGEC

SEQ ID NO: 89 - protein, 214 aa, Artificial Sequence
  humanized antibody light chain KB
DIQMTQSPSSVSASVGDRVTITCRASQDISSYLNWYQQKPGKAPKLLIYYTSRLHSGVPSRFSGSGSGTDYTLTISSLQPEDFASYFCQQLNTLPWTFGGGTKVEMERTVAAPSVFIFPPSDEQLKSGTASVVCLLNNFYPREAKVQWKVDNALQSGNSQESVTEQDSKDSTYSLSSTLTLSKADYEKHKVYACEVTHQGLSSPVTKSFNRGEC

SEQ ID NO: 90 - protein, 214 aa, Artificial Sequence
  humanized antibody light chain KC
DIQMTQSPSSVSASVGDRVTITCRASQDISSYLNWYQQKPGKAVKLLIYYTSRLHSGVPSRFSGSGSGTDYTLTISSLQPEDFASYFCQQLNTLPWTFGGGTKVEMERTVAAPSVFIFPPSDEQLKSGTASVVCLLNNFYPREAKVQWKVDNALQSGNSQESVTEQDSKDSTYSLSSTLTLSKADYEKHKVYACEVTHQGLSSPVTKSFNRGEC

SEQ ID NO: 91 - protein, 214 aa, Artificial Sequence
  humanized antibody light chain KD
DIQMTQSPSSVSASVGDRVTITCRASQDISSYLNWYQQKPGKAPKLLIYYTSRLHSGVPSRFSGSGSGTDFTLTISSLQPEDFATYFCQQLNTLPWTFGGGTKVEMERTVAAPSVFIFPPSDEQLKSGTASVVCLLNNFYPREAKVQWKVDNALQSGNSQESVTEQDSKDSTYSLSSTLTLSKADYEKHKVYACEVTHQGLSSPVTKSFNRGEC

SEQ ID NO: 92 - protein, 214 aa, Artificial Sequence
  humanized antibody light chain KE
DIQMTQSPSSVSASVGDRVTITCRASQDISSYLNWYQQKPGKAVKLLIYYTSRLHSGVPSRFSGSGSGTDFTLTISSLQPEDFASYFCQQLNTLPWTFGGGTKVEMERTVAAPSVFIFPPSDEQLKSGTASVVCLLNNFYPREAKVQWKVDNALQSGNSQESVTEQDSKDSTYSLSSTLTLSKADYEKHKVYACEVTHQGLSSPVTKSFNRGEC

SEQ ID NO: 93 - protein, 214 aa, Artificial Sequence
  humanized antibody light chain KF
DIQMTQSPSSVSASVGDRVTITCRASQDISSYLNWYQQKPGKAVKLLIYYTSRLHSGVPSRFSGSGSGTDFTLTISSLQPEDFATYFCQQLNTLPWTFGGGTKVEMERTVAAPSVFIFPPSDEQLKSGTASVVCLLNNFYPREAKVQWKVDNALQSGNSQESVTEQDSKDSTYSLSSTLTLSKADYEKHKVYACEVTHQGLSSPVTKSFNRGEC

SEQ ID NO: 94 - protein, 214 aa, Artificial Sequence
  humanized antibody light chain KG
DIQMTQSPSSVSASVGDRVTITCRASQDISSYLNWYQQKPGKAVKLLIYYTSRLHSGVPSRFSGSGSGTDYTLTISSLQPEDFATYFCQQLNTLPWTFGGGTKVEMERTVAAPSVFIFPPSDEQLKSGTASVVCLLNNFYPREAKVQWKVDNALQSGNSQESVTEQDSKDSTYSLSSTLTLSKADYEKHKVYACEVTHQGLSSPVTKSFNRGEC

SEQ ID NO: 95 - protein, 116 aa, Artificial Sequence
  humanized antibody heavy chain
EVQLVESGGGLVQPGRSLRLSCTASGFTFSDAWMDWVRQAPGKGLEWVAEIRSKANNHATYYAESVKGRFTISRDDSKSIVYLQMNSLRTEDTALYYCTRRDGAYWGKGTTVTVSS

SEQ ID NO: 96 - protein, 107 aa, Artificial Sequence
  humanized antibody light chain
DIQMTQSPSSVSASVGDRVTITCRASQDISSYLNWYQQKPGKAPKLLIYYTSRLHSGVPSRFSGSGSGTDFTLTISSLQPEDFASYFCQQLNTLPWTFGGGTKVEME

SEQ ID NO: 97 - protein, 14 aa, Artificial Sequence
  Description of Artificial Sequence: Synthetic peptide
TGTSSSVGDSIYVS

SEQ ID NO: 98 - protein, 7 aa, Artificial Sequence
  Description of Artificial Sequence: Synthetic peptide
DVTKRPS

SEQ ID NO: 99 - protein, 9 aa, Artificial Sequence
  Description of Artificial Sequence: Synthetic peptide
CSYAGTDTL

SEQ ID NO: 100 - protein, 5 aa, Artificial Sequence
  Description of Artificial Sequence: Synthetic peptide
SHGIS

SEQ ID NO: 101 - protein, 17 aa, Artificial Sequence
  Description of Artificial Sequence: Synthetic peptide
WISPYSGNTNYAQKLQG

SEQ ID NO: 102 - protein, 11 aa, Artificial Sequence
  Description of Artificial Sequence: Synthetic peptide
VGSGPYYYMDV

SEQ ID NO: 103 - protein, 9 aa, Artificial Sequence
  Description of Artificial Sequence: Synthetic peptide
YSYAGTDTL

SEQ ID NO: 104 - protein, 9 aa, Artificial Sequence
  Description of Artificial Sequence: Synthetic peptide
FSYAGTDTL

SEQ ID NO: 105 - protein, 9 aa, Artificial Sequence
  Description of Artificial Sequence: Synthetic peptide
HSYAGTDTL

SEQ ID NO: 106 - protein, 9 aa, Artificial Sequence
  Description of Artificial Sequence: Synthetic peptide
LSYAGTDTL

SEQ ID NO: 107 - protein, 9 aa, Artificial Sequence
  Description of Artificial Sequence: Synthetic peptide
VSYAGTDTL

SEQ ID NO: 108 - protein, 9 aa, Artificial Sequence
  Description of Artificial Sequence: Synthetic peptide
ISYAGTDTL

SEQ ID NO: 109 - protein, 9 aa, Artificial Sequence
  Description of Artificial Sequence: Synthetic peptide
KSYAGTDTL